European Patent Application EP 4 768 498 A1, published July 1, 2026. Title: PEPTIDES, KITS FOR DOROPLET FORMATION, METHODS FOR FORMING DOROPLETS, METHODS FOR CONCENTRATING HYDROPHOBIC SUBSTANCES, AND METHODS FOR PROTEIN FOLDING. Applicant: 国立大学法人東京農工大学. The sequence listing filed with the application follows.

SEQUENCE LISTING (5 sequences)

SEQ ID NO: 1 - protein, 5 aa, synthetic construct
  VARIANT 4: note = X indicates any amino acid residue other than a proline residue
VPGXG

SEQ ID NO: 2 - protein, 22 aa, synthetic construct
  VARIANT 6: note = X indicates any amino acid residue other than a proline residue
  VARIANT 11: note = X indicates any amino acid residue other than a proline residue
  VARIANT 16: note = X indicates any amino acid residue other than a proline residue
  VARIANT 21: note = X indicates any amino acid residue other than a proline residue
LLVPGXGVPGXGVPGXGVPGXG

SEQ ID NO: 3 - protein, 22 aa, synthetic construct
LLVPGVGVPGVGVPGVGVPGVG

SEQ ID NO: 4 - protein, 25 aa, synthetic construct
  VARIANT 6: note = X indicates any amino acid residue other than a proline residue
  VARIANT 11: note = X indicates any amino acid residue other than a proline residue
  VARIANT 19: note = X indicates any amino acid residue other than a proline residue
  VARIANT 24: note = X indicates any amino acid residue other than a proline residue
LLVPGXGVPGXGCHCVPGXGVPGXG

SEQ ID NO: 5 - protein, 26 aa, synthetic construct
LLVPGVGVPGVGCGHCVPGVGVPGVG